European Patent Specification EP 4 090 971 B1, published February 26, 2025. Title: Method for separation of sperm with undamaged intact heads from sperm with damaged heads and somatic cells. Applicant: Biotechnologicky ustav AV CR, v. v. i. The sequence listing filed with the application follows.

SEQUENCE LISTING (1 sequence)

SEQ ID NO: 1 - protein, 14 aa, artificial
  immunization peptide
PFEAMELKGTPKLY